European Patent Specification EP 3 453 392 B1, published October 22, 2025. Title: Brigatinib and its analogs overcome registance in EGFR-mutated non-small-cell lung cancer. Applicant: Japanese Foundation for Cancer Research. The sequence listing filed with the application follows.

SEQUENCE LISTING (4 sequences)

SEQ ID NO: 1 - DNA, 32 bp, Artificial Sequence
  PCR primer
ccgtgcagctcatcatccagctcatgcccttc

SEQ ID NO: 2 - DNA, 32 bp, Artificial Sequence
  PCR primer
gaagggcatgagctgcatgatgagctgcacgg

SEQ ID NO: 3 - DNA, 28 bp, Artificial Sequence
  PCR primer
catgcccttcggctccctcctggagcta

SEQ ID NO: 4 - DNA, 27 bp, Artificial Sequence
  PCR primer
tagtccaggagggagccgaagggcatg